European Patent Application EP 4 206 231 A1, published July 5, 2023. Title: Recombinant RSV Antigens. Applicant: ID Biomedical Corporation of Quebec. Application EP, filed December 23, 2008. The sequence listing filed with the application follows.

SEQUENCE LISTING (16 sequences)

SEQ ID NO: 1 - DNA, 1697 bp, respiratory syncytial virus
  source 1..1697: mol_type = genomic DNA
atggagttgctaatcctcaaagcaaatgcaattaccacaatcctcactgcagtcacatttgttttgcttctggtcaaaacatcactgaagaattttatcaatcaacatgcagtgcagtagcaaaggctatcttagtgctctgagaactggttggtataccagtgttataactatagattaagtaatatcaaggaaaataagtgtaatggaacagatgctaaggtaaaattgataaacaagaattagataaatataaaaatgctgtaacagaattgcagttgctcatgcaaagcacccagcaacaaacaatcgagccagaagagaactaccaaggtttatgaattatacactcaaaatgccaaaaaaaccaatgtaacattaagcaagaaaaggaaaagaagatttcttggtttttgttaggtgttggatctgcaatcgccagtggcgttgctgtatctaaggtcctgcacctgaaggggaagtgaacaagatcaaaagtgctctactatccacaaacaaggctgtagtcagttatcaaatggagttagtgtcttaaccagcaaagtgttagacctcaaaaactatatagaaaacaattgttacctattgtgaacaagcaaagctgcagcatatcaaatatagcaactgtatagagttccaacaaaagaacaacagactactagagattaccagggaatttagtgttaagcaggtgtaactacacctgtaagcacttacatgttaactaatagtgaattattgtcattatcaatgatatgcctataacaaatgatcagaaaaagttaatgtccaacaatgttcaaatgttagacagcaaagttactctatcatgtccataataaaagaggaagtcttagcatatgtgtacaattaccactatatggtgttatagatacaccctgttggaaactacacacatccccctatgtacaaccaacacaaaagaagggtccaacatctgtttaacaagaactgacagaggtggtactgtgacaatgcaggatcagtatctttcttcccacaagctgaaacatgtaaagtcaatcaaatcgagtattttgtgacacaatgaacagtttaacattaccaagtgaagtaaactctgcaatgttgacatattcaaccccaaatatgattgtaaaattatgacttcaaaaacgatgtaagcagctccgttatcacatctctaggagccattgtgtcatgctatggcaaaacaaatgtacagcatccaataaaaatcgtggaatcataaagacattttctaacgggtgcgatatgtatcaaataaaggggtggacactgtgtctgtaggtaacacattatattatgtaaaaagcaagaaggtaaaagtctctatgtaaaaggtgaaccaataataaatttctatgacccttagtattcccctctgatgaatttgatgcatcaatatctcaagtcaacgagaagattaacagagcctagcatttattcgtaaatccgatgaattattacataatgtaaatgctggtaatccaccataaatatcatgataactactataattatagtgattatagtaatattgttatcttaattgctgttggactgctcttatactgtaaggccagaagcacaccagtcacactaagaaagatcaactgagtggtataaataatattgcatttagtaactaa

SEQ ID NO: 2 - protein, 574 aa, respiratory syncytial virus
MELLILKANAITTILTAVTFCFASGQNITEEFYQSTCSAVSKGYLSALRTGWYTSVITIELSNIKENKCNGTDAKVKLIKQELDKYKNAVTELQLLMQSTPATNNRARRELPRFMNYTLNNAKKTNVTLSKKRKRRFLGFLLGVGSAIASGVAVSKVLHLEGEVNKIKSALLSTNKAVVSLSNGVSVLTSKVLDLKNYIDKQLLPIVNKQSCSISNIATVIEFQQKNNRLLEITREFSVNAGVTTPVSTYMLTNSELLSLINDMPITNDQKKLMSNNVQIVRQQSYSIMSIIKEEVLAYVVQLPLYGVIDTPCWKLHTSPLCTTNTKEGSNICLTRTDRGWYCDNAGSVSFFPQAETCKVQSNRVFCDTMNSLTLPSEVNLCNVDIFNPKYDCKIMTSKTDVSSSVITSLGAIVSCYGKTKCTASNKNRGIIKTFSNGCDYVSNKGVDTVSVGNTLYYVNKQEGKSLYVKGEPIINFYDPLVFPSDEFDASISQVNEKINQSLAFIRKSDELLHNVNAGKSTINIMITTIIIVIIVILLSLIAVGLLLYCKARSTPVTLSKDQLSGINNIAFSN

SEQ ID NO: 3 - DNA, 897 bp, respiratory syncytial virus
  source 1..897: mol_type = genomic DNA
atgtccaaaaacaaggaccaacgcaccgctaagacactagaaaagacctgggacactctcaatcatttattattcatatcatcgggcttatataagttaaatcttaaatctatagcacaaatcacattatccattctggcaatgataatctcaacttcacttataattacagccatcatattcatagcctcggcaaaccacaaagtcacactaacaactgcaatcatacaagatgcaacaagccagatcaagaacacaaccccaacatacctcactcaggatcctcagcttggaatcagcttctccaatctgtctgaaattacatcacaaaccaccaccatactagcttcaacaacaccaggagtcaagtcaaacctgcaacccacaacagtcaagactaaaaacacaacaacaacccaaacacaacccagcaagcccactacaaaacaacgccaaaacaaaccaccaaacaaacccaataatgattttcacttcgaagtgtttaactttgtaccctgcagcatatgcagcaacaatccaacctgctgggctatctgcaaaagaataccaaacaaaaaaccaggaaagaaaaccaccaccaagcctacaaaaaaaccaaccttcaagacaaccaaaaaagatctcaaacctcaaaccactaaaccaaaggaagtacccaccaccaagcccacagaagagccaaccatcaacaccaccaaaacaaacatcacaactacactgctcaccaacaacaccacaggaaatccaaaactcacaagtcaaatggaaaccttccactcaacctcctccgaaggcaatctaagcccttctcaagtctccacaacatccgagcacccatcacaaccctcatctccacccaacacaacacgccagtag

SEQ ID NO: 4 - protein, 298 aa, respiratory syncytial virus
MSKNKDQRTAKTLEKTWDTLNHLLFISSGLYKLNLKSIAQITLSILAMIISTSLIITAIIFIASANHKVTLTTAIIQDATSQIKNTTPTYLTQDPQLGISFSNLSEITSQTTTILASTTPGVKSNLQPTTVKTKNTTTTQTQPSKPTTKQRQNKPPNKPNNDFHFEVFNFVPCSICSNNPTCWAICKRIPNKKPGKKTTTKPTKKPTFKTTKKDLKPQTTKPKEVPTTKPTEEPTINTTKTNITTTLLTNNTTGNPKLTSQMETFHSTSSEGNLSPSQVSTTSEHPSQPSSPPNTTRQ

SEQ ID NO: 5 - DNA, 1566 bp, synthetic construct
  misc_feature 1..1566: note = Recombinant PreF polynucleotide
  source 1..1566: mol_type = other DNA
aagcttgccaccatggagctgctgatcctgaaaaccaacgccatcaccgccatcctggccgccgtgaccctgtgcttcgcctcctcccagaacatcaccgaggagttctaccagtccacctgctccgccgtgtccaagggctacctgtccgccctgcggaccggctggtacacctccgtgatcaccatcgagctgtccaacatcaaggaaaacaagtgcaacggcaccgacgccaaggtgaagctgatcaagcaggagctggacaagtacaagagcgccgtgaccgaactccagctgctgatgcagtccacccctgccaccaacaacaagtttctgggcttcctgctgggcgtgggctccgccatcgcctccggcatcgccgtgagcaaggtgctgcacctggagggcgaggtgaacaagatcaagagcgccctgctgtccaccaacaaggccgtggtgtccctgtccaacggcgtgtccgtgctgacctccaaggtgctggatctgaagaactacatcgacaagcagctgctgcctatcgtgaacaagcagtcctgctccatctccaacatcgagaccgtgatcgagttccagcagaagaacaaccggctgctggagatcacccgcgagttctccgtgaacgccggcgtgaccacccctgtgtccacctacatgctgaccaactccgagctgctgtccctgatcaacgacatgcctatcaccaacgaccagaaaaaactgatgtccaacaacgtgcagatcgtgcggcagcagtcctacagcatcatgagcatcatcaaggaagaggtgctggcctacgtggtgcagctgcctctgtacggcgtgatcgacaccccttgctggaagctgcacacctcccccctgtgcaccaccaacaccaaggagggctccaacatctgcctgacccggaccgaccggggctggtactgcgacaacgccggctccgtgtccttcttccctctggccgagacctgcaaggtgcagtccaaccgggtgttctgcgacaccatgaactccctgaccctgccttccgaggtgaacctgtgcaacatcgacatcttcaaccccaagtacgactgcaagatcatgaccagcaagaccgacgtgtcctccagcgtgatcacctccctgggcgccatcgtgtcctgctacggcaagaccaagtgcaccgcctccaacaagaaccggggaatcatcaagaccttctccaacggctgcgactacgtgtccaataagggcgtggacaccgtgtccgtgggcaacacactgtactacgtgaataagcaggagggcaagagcctgtacgtgaagggcgagcctatcatcaacttctacgaccctctggtgttcccttccgacgagttcgacgcctccatcagccaggtgaacgagaagatcaaccagtccctggccttcatccggaagtccgacgagaagctgcataacgtggaggacaagatcgaggagatcctgtccaaaatctaccacatcgagaacgagatcgcccggatcaagaagctgatcggcgaggcctgataatctaga

SEQ ID NO: 6 - protein, 514 aa, synthetic construct
  REGION 1..514: note = Recombinant PreF Antigen
MELLILKTNAITAILAAVTLCFASSQNITEEFYQSTCSAVSKGYLSALRTGWYTSVITIELSNIKENKCNGTDAKVKLIKQELDKYKSAVTELQLLMQSTPATNNKFLGFLLGVGSAIASGIAVSKVLHLEGEVNKIKSALLSTNKAVVSLSNGVSVLTSKVLDLKNYIDKQLLPIVNKQSCSISNIETVIEFQQKNNRLLEITREFSVNAGVTTPVSTYMLTNSELLSLINDMPITNDQKKLMSNNVQIVRQQSYSIMSIIKEEVLAYVVQLPLYGVIDTPCWKLHTSPLCTTNTKEGSNICLTRTDRGWYCDNAGSVSFFPLAETCKVQSNRVFCDTMNSLTLPSEVNLCNIDIFNPKYDCKIMTSKTDVSSSVITSLGAIVSCYGKTKCTASNKNRGIIKTFSNGCDYVSNKGVDTVSVGNTLYYVNKQEGKSLYVKGEPIINFYDPLVFPSDEFDASISQVNEKINQSLAFIRKSDEKLHNVEDKIEEILSKIYHIENEIARIKKLIGEA

SEQ ID NO: 7 - DNA, 1855 bp, synthetic construct
  misc_feature 1..1855: note = Chimeric PreF-G Antigen polynucleotide seqeunce
  source 1..1855: mol_type = other DNA
aagcttgccaccatggagctgctgatcctcaagaccaacgccatcaccgccatcctggccgccgtgaccctgtgcttcgcctcctcccagaacatcaccgaagagttctaccagtccacctgctccgccgtgtccaagggctacctgtccgccctgcggaccggctggtacacctccgtgatcaccatcgagctgtccaacatcaaagaaaacaagtgcaacggcaccgacgccaaggtcaagctgatcaagcaggaactggacaagtacaagagcgccgtgaccgaactccagctgctgatgcagtccacccctgccaccaacaacaagaagtttctgggcttcctgctgggcgtgggctccgccatcgcctccggcatcgccgtgagcaaggtgctgcacctggagggcgaggtgaacaagatcaagagcgccctgctgtccaccaacaaggccgtggtgtccctgtccaacggcgtgtccgtgctgacctccaaggtgctggatctgaagaactacatcgacaagcagctgctgcctatcgtgaacaagcagtcctgctccatctccaacatcgagaccgtgatcgagttccagcagaagaacaaccggctgctggagatcacccgcgagttctccgtgaacgccggcgtgaccacccctgtgtccacctacatgctgacaaactccgagctgctctccctgatcaacgacatgcctatcaccaacgaccaaaaaaagctgatgtccaacaacgtgcagatcgtgcggcagcagtcctacagcatcatgagcatcatcaaggaagaagtcctggcctacgtcgtgcagctgcctctgtacggcgtgatcgacaccccttgctggaagctgcacacctcccccctgtgcaccaccaacaccaaagagggctccaacatctgcctgacccggaccgaccggggctggtactgcgacaacgccggctccgtgtccttcttccctctggccgagacctgcaaggtgcagtccaaccgggtgttctgcgacaccatgaactccctgaccctgccttccgaggtgaacctgtgcaacatcgacatcttcaaccccaagtacgactgcaagatcatgaccagcaagaccgacgtgtcctccagcgtgatcacctccctgggcgccatcgtgtcctgctacggcaagaccaagtgcaccgcctccaacaagaaccggggaatcatcaagaccttctccaacggctgcgactacgtgtccaataagggcgtggacaccgtgtccgtgggcaacacactgtactacgtgaataagcaggaaggcaagagcctgtacgtgaagggcgagcctatcatcaacttctacgaccctctggtgttcccttccgacgagttcgacgcctccatcagccaggtcaacgagaagatcaaccagtccctggccttcatccggaagtccgacgagaagctgcataacgtggaggacaagatcgaagagatcctgtccaaaatctaccacatcgagaacgagatcgcccggatcaagaagctgatcggcgaggctggcggctctggcggcagcggcggctccaagcagcggcagaacaagcctcctaacaagcccaacaacgacttccacttcgaggtgttcaacttcgtgccttgctccatctgctccaacaaccctacctgctgggccatctgcaagagaatccccaacaagaagcctggcaagaaaaccaccaccaagcctaccaagaagcctaccttcaagaccaccaagaaggaccacaagcctcagaccacaaagcctaaggaagtgccaaccaccaagcaccaccaccatcaccactgataatcta

SEQ ID NO: 8 - protein, 605 aa, synthetic construct
  REGION 1..605: note = Chimeric PreF-G polypeptide
MELLILKTNAITAILAAVTLCFASSQNITEEFYQSTCSAVSKGYLSALRTGWYTSVITIELSNIKENKCNGTDAKVKLIKQELDKYKSAVTELQLLMQSTPATNNKKFLGFLLGVGSAIASGIAVSKVLHLEGEVNKIKSALLSTNKAVVSLSNGVSVLTSKVLDLKNYIDKQLLPIVNKQSCSISNIETVIEFQQKNNRLLEITREFSVNAGVTTPVSTYMLTNSELLSLINDMPITNDQKKLMSNNVQIVRQQSYSIMSIIKEEVLAYVVQLPLYGVIDTPCWKLHTSPLCTTNTKEGSNICLTRTDRGWYCDNAGSVSFFPLAETCKVQSNRVFCDTMNSLTLPSEVNLCNIDIFNPKYDCKIMTSKTDVSSSVITSLGAIVSCYGKTKCTASNKNRGIIKTFSNGCDYVSNKGVDTVSVGNTLYYVNKQEGKSLYVKGEPIINFYDPLVFPSDEFDASISQVNEKINQSLAFIRKSDEKLHNVEDKIEEILSKIYHIENEIARIKKLIGEAGGSGGSGGSKQRQNKPPNKPNNDFHFEVFNFVPCSICSNNPTCWAICKRIPNKKPGKKTTTKPTKKPTFKTTKKDHKPQTTKPKEVPTTK

SEQ ID NO: 9 - DNA, 1834 bp, synthetic construct
  misc_feature 1..1834: note = Chimeric PreF-G polynucleotide
  source 1..1834: mol_type = other DNA
aagcttgccaccatggagctgctgatcctcaagaccaacgccatcaccgccatcctggccgccgtgaccctgtgcttcgcctcctcccagaacatcaccgaagagttctaccagtccacctgctccgccgtgtccaagggctacctgtccgccctgcggaccggctggtacacctccgtgatcaccatcgagctgtccaacatcaaagaaaacaagtgcaacggcaccgacgccaaggtcaagctgatcaagcaggaactggacaagtacaagagcgccgtgaccgaactccagctgctgatgcagtccacccctgccaccaacaacaagaagtttctgggcttcctgctgggcgtgggctccgccatcgcctccggcatcgccgtgagcaaggtgctgcacctggagggcgaggtgaacaagatcaagagcgccctgctgtccaccaacaaggccgtggtgtccctgtccaacggcgtgtccgtgctgacctccaaggtgctggatctgaagaactacatcgacaagcagctgctgcctatcgtgaacaagcagtcctgctccatctccaacatcgagaccgtgatcgagttccagcagaagaacaaccggctgctggagatcacccgcgagttctccgtgaacgccggcgtgaccacccctgtgtccacctacatgctgacaaactccgagctgctctccctgatcaacgacatgcctatcaccaacgaccaaaaaaagctgatgtccaacaacgtgcagatcgtgcggcagcagtcctacagcatcatgagcatcatcaaggaagaagtcctggcctacgtcgtgcagctgcctctgtacggcgtgatcgacaccccttgctggaagctgcacacctcccccctgtgcaccaccaacaccaaagagggctccaacatctgcctgacccggaccgaccggggctggtactgcgacaacgccggctccgtgtccttcttccctctggccgagacctgcaaggtgcagtccaaccgggtgttctgcgacaccatgaactccctgaccctgccttccgaggtgaacctgtgcaacatcgacatcttcaaccccaagtacgactgcaagatcatgaccagcaagaccgacgtgtcctccagcgtgatcacctccctgggcgccatcgtgtcctgctacggcaagaccaagtgcaccgcctccaacaagaaccggggaatcatcaagaccttctccaacggctgcgactacgtgtccaataagggcgtggacaccgtgtccgtgggcaacacactgtactacgtgaataagcaggaaggcaagagcctgtacgtgaagggcgagcctatcatcaacttctacgaccctctggtgttcccttccgacgagttcgacgcctccatcagccaggtcaacgagaagatcaaccagtccctggccttcatccggaagtccgacgagaagctgcataacgtggaggacaagatcgaagagatcctgtccaaaatctaccacatcgagaacgagatcgcccggatcaagaagctgatcggcgaggctggcggcaagcagcggcagaacaagcctcctaacaagcccaacaacgacttccacttcgaggtgttcaacttcgtgccttgctccatctgctccaacaaccctacctgctgggccatctgcaagagaatccccaacaagaagcctggcaagaaaaccaccaccaagcctaccaagaagcctaccttcaagaccaccaagaaggaccacaagcctcagaccacaaagcctaaggaagtgccaaccaccaagcaccaccaccatcaccactgataatcta

SEQ ID NO: 10 - protein, 598 aa, synthetic construct
  REGION 1..598: note = Chimeric PreF-G polypeptide
MELLILKTNAITAILAAVTLCFASSQNITEEFYQSTCSAVSKGYLSALRTGWYTSVITIELSNIKENKCNGTDAKVKLIKQELDKYKSAVTELQLLMQSTPATNNKKFLGFLLGVGSAIASGIAVSKVLHLEGEVNKIKSALLSTNKAVVSLSNGVSVLTSKVLDLKNYIDKQLLPIVNKQSCSISNIETVIEFQQKNNRLLEITREFSVNAGVTTPVSTYMLTNSELLSLINDMPITNDQKKLMSNNVQIVRQQSYSIMSIIKEEVLAYVVQLPLYGVIDTPCWKLHTSPLCTTNTKEGSNICLTRTDRGWYCDNAGSVSFFPLAETCKVQSNRVFCDTMNSLTLPSEVNLCNIDIFNPKYDCKIMTSKTDVSSSVITSLGAIVSCYGKTKCTASNKNRGIIKTFSNGCDYVSNKGVDTVSVGNTLYYVNKQEGKSLYVKGEPIINFYDPLVFPSDEFDASISQVNEKINQSLAFIRKSDEKLHNVEDKIEEILSKIYHIENEIARIKKLIGEAGGKQRQNKPPNKPNNDFHFEVFNFVPCSICSNNPTCWAICKRIPNKKPGKKTTTKPTKKPTFKTTKKDHKPQTTKPKEVPTTK

SEQ ID NO: 11 - protein, 28 aa, synthetic construct
  REGION 1..28: note = Isoleucine substituted GCN4 leucine zipper
EDKIEEILSKIYHIENEIARIKKLIGEA

SEQ ID NO: 12 - DNA, 1563 bp, synthetic construct
  misc_feature 1..1563: note = Codon optimized PreF nucleotide sequence
  source 1..1563: mol_type = other DNA
atggagctgcccatcctgaagaccaacgccatcaccaccatcctcgccgccgtgaccctgtgcttcgccagcagccagaacatcacggaggagttctaccagagcacgtgcagcgccgtgagcaagggctacctgagcgcgctgcgcacgggctggtacacgagcgtgatcacgatcgagctgagcaacatcaaggagaacaagtgcaacggcacggacgcgaaggtgaagctgatcaagcaggagctggacaagtacaagagcgcggtgacggagctgcagctgctgatgcagagcacgccggcgacgaacaacaagttcctcggcttcctgctgggcgtgggcagcgcgatcgcgagcggcatcgccgtgagcaaggtgctgcacctggagggcgaggtgaacaagatcaagtccgcgctgctgagcacgaacaaggcggtcgtgagcctgagcaacggcgtgagcgtgctgacgagcaaggtgctcgacctgaagaactacatcgacaagcagctgctgccgatcgtgaacaagcagagctgcagcatcagcaacatcgagaccgtgatcgagttccagcagaagaacaaccgcctgctggagatcacgcgggagttctccgtgaacgcaggcgtgacgacgcccgtgtctacgtacatgctgacgaacagcgagctgctcagcctgatcaacgacatgccgatcacgaacgaccagaagaagctgatgagcaacaacgtgcagatcgtgcgccagcagagctacagcatcatgagcatcatcaaggaggaggtgctggcatacgtggtgcagctgccgctgtacggcgtcatcgacacgccctgctggaagctgcacacgagcccgctgtgcacgaccaacacgaaggagggcagcaacatctgcctgacgcggacggaccggggctggtactgcgacaacgcgggcagcgtgagcttcttcccgctcgcggagacgtgcaaggtgcagagcaaccgcgtcttctgcgacacgatgaacagcctgacgctgccgagcgaggtgaacctgtgcaacatcgacatcttcaacccgaagtacgactgcaagatcatgacgagcaagaccgatgtcagcagcagcgtgatcacgagcctcggcgcgatcgtgagctgctacggcaagacgaagtgcacggcgagcaacaagaaccgcggcatcatcaagacgttcagcaacggctgcgactatgtgagcaacaagggcgtggacactgtgagcgtcggcaacacgctgtactacgtgaacaagcaggagggcaagagcctgtacgtgaagggcgagccgatcatcaacttctacgacccgctcgtgttcccgagcgacgagttcgacgcgagcatcagccaagtgaacgagaagatcaaccagagcctggcgttcatccgcaagagcgacgagaagctgcacaacgtggaggacaagatcgaggagatcctgagcaagatctaccacatcgagaacgagatcgcgcgcatcaagaagctgatcggcgaggcgcatcatcaccatcaccattga

SEQ ID NO: 13 - DNA, 1685 bp, synthetic construct
  misc_feature 1..1685: note = PreF polynucleotide sequence with intron
  source 1..1685: mol_type = other DNA
atggagctgctgatcctgaaaaccaacgccatcaccgccatcctggccgccgtgaccctgtgcttcgcctcctcccagaacatcaccgaggagttctaccagtccacctgctccgccgtgtccaagggctacctgtccgccctgcggaccggctggtacacctccgtgatcaccatcgagctgtccaacatcaaggaaaacaagtgcaacggcaccgacgccaaggtgaagctgatcaagcaggagctggacaagtacaagagcgccgtgaccgaactccagctgctgatgcagtccacccctgccaccaacaacaagtttctgggcttcctgctgggcgtgggctccgccatcgcctccggcatcgccgtgagcaaggtacgtgtcgggacttgtgttcccctttttttaataaaaagttatatctttaatgttatatacatatttcctgtatgtgatccatgtgcttatgactttgtttatcatgtgtttaggtgctgcacctggagggcgaggtgaacaagatcaagagcgccctgctgtccaccaacaaggccgtggtgtccctgtccaacggcgtgtccgtgctgacctccaaggtgctggatctgaagaactacatcgacaagcagctgctgcctatcgtgaacaagcagtcctgctccatctccaacatcgagaccgtgatcgagttccagcagaagaacaaccggctgctggagatcacccgcgagttctccgtgaacgccggcgtgaccacccctgtgtccacctacatgctgaccaactccgagctgctgtccctgatcaacgacatgcctatcaccaacgaccagaaaaaactgatgtccaacaacgtgcagatcgtgcggcagcagtcctacagcatcatgagcatcatcaaggaagaggtgctggcctacgtggtgcagctgcctctgtacggcgtgatcgacaccccttgctggaagctgcacacctcccccctgtgcaccaccaacaccaaggagggctccaacatctgcctgacccggaccgaccggggctggtactgcgacaacgccggctccgtgtccttcttccctctggccgagacctgcaaggtgcagtccaaccgggtgttctgcgacaccatgaactccctgaccctgccttccgaggtgaacctgtgcaacatcgacatcttcaaccccaagtacgactgcaagatcatgaccagcaagaccgacgtgtcctccagcgtgatcacctccctgggcgccatcgtgtcctgctacggcaagaccaagtgcaccgcctccaacaagaaccggggaatcatcaagaccttctccaacggctgcgactacgtgtccaataagggcgtggacaccgtgtccgtgggcaacacactgtactacgtgaataagcaggagggcaagagcctgtacgtgaagggcgagcctatcatcaacttctacgaccctctggtgttcccttccgacgagttcgacgcctccatcagccaggtgaacgagaagatcaaccagtccctggccttcatccggaagtccgacgagaagctgcataacgtggaggacaagatcgaggagatcctgtccaaaatctaccacatcgagaacgagatcgcccggatcaagaagctgatcggcgaggccggaggtcaccaccaccatcaccactga

SEQ ID NO: 14 - protein, 9 aa, synthetic construct
  REGION 1..9: note = Synthetic linker peptide
GGSGGSGGS

SEQ ID NO: 15 - protein, 4 aa, synthetic construct
  REGION 1..4: note = Furin cleavage consensus motif
RARR

SEQ ID NO: 16 - protein, 4 aa, synthetic construct
  REGION 1..4: note = Furin cleavage consensus motif
RKRR